European Patent Application EP 4 269 558 A1, published November 1, 2023. Title: CULTURE MATERIAL AND USE THEREOF. Applicant: MITSUI CHEMICALS, INC. The sequence listing filed with the application follows.

SEQUENCE LISTING (6 sequences)

SEQ ID NO: 1 - DNA, 22 bp, Artificial
  GAPDH Fw
attgccctcaacgaccactttg

SEQ ID NO: 2 - DNA, 22 bp, Artificial
  GAPDH Rv
tcttcctcttgtgctcttgctg

SEQ ID NO: 3 - DNA, 20 bp, Artificial
  MYL2 Fw
aggctccgggtccaattaac

SEQ ID NO: 4 - DNA, 20 bp, Artificial
  MYL2 Rv
ttgccttcagggtcaaacac

SEQ ID NO: 5 - DNA, 22 bp, Artificial
  MYL7 Fw
tcagctgtatcgaccagaatcg

SEQ ID NO: 6 - DNA, 22 bp, Artificial
  MYL7 Rv
aggaagacggtgaagttgatgg